European Patent Application EP 4 140 293 A1, published March 1, 2023. Title: TOBACCO PLANT AND METHOD FOR MANUFACTURING SAME. Applicant: JAPAN TOBACCO INC. The sequence listing filed with the application follows.

SEQUENCE LISTING (23 sequences)

SEQ ID NO: 1 - protein, 600 aa, Nicotiana tabacum
MDAFSSTFLSTLSQHPKSLLSPNYSPNTSSSPSLKVSSVRIEERPQTTTRTKPQEKPTPSPYTAPKDTPKRQLPTKSITPQKTVEPPFPSVIFNAFDDFVNTFIDPPLKPSVDPKYILSNNFAPVEELPPTECEVVVGSLPPCLDGAYIRNGPNPQYLPRGPYHLFDGDGMLHSIKISQGKATLCSRYVKTYKYTIEREAGSPVLPNVFSGFNGLTASAARGAITAARAIAGQFNPTNGIGLANTSLALFGGKLFALGESDLPYAVKLAPDGDIITLGRYDFDGKLFMSMTAHPKIDPDTNEAFAFRYGPMPPFLTYFRIEPSGTKTPDVPIFSMTRPSFLHDFAITKKYAIFSDIQIGMNPLEFIAGGSPVSSDSGKIPRLGVIPRYAKDESEMKWFDVPGFNIVHAINAWDEDDGDTIVMVAPNILSVEHTLERMDMIHASVEKVKIDLKSGMVSRHPVSTRNLDFGVINPAYVGKKNKYVYAAIGDPMPKIAGIAKLDVSVAEADRRDCIVGCRLFGEGCFGGEPYFVAKNPNNSVADEDDGYVVSYVHNEKTGESRFLVMDAKSPNLDIVAAVKLPRRVPYGFHGLFVREIDLSKL

SEQ ID NO: 2 - protein, 600 aa, Nicotiana tabacum
MDAFSSTFLSTLSLHPKSLLSPNYSPNTSSSLALKVSSVRIEERPQTTTRTKPQEKPTPSPYTPPKDTPKRQLPTKSTTTKKTVKPSFPSVIFNAFDDFVNTFIDPPLKPSVDPKYILSNNFAPVDELPPTECEVVVGSLPPCLDGAYIRNGPNPQYLPRGPYHLFDGDGMLHCIKISQGKATLCSRYVKTYKYIIEREAGSPVIPNVFSGFNGLTASAARGAITAARAIAGQFNPTNGIGLANTSLALFGGKLFALGESDLPYAVKLAPDGDIITLGRYDFDGKLFMSMTAHPKIDPDTNEAFAFRYGPMPPFLTYFRIEPNGTKTPDVPIFSMTRPSFLHDFAITKKYAIFSDIQIGMNPLEFITGGSPVSSDSGKVPRLGVIPRYAKDESEMRWFDVPGFNIVHAINAWDEDDGDTIVMVAPNILSVEHTLERMDMIHASVEKVKIDLKSGMVSRHPVSTRNLDFGVINPAYVGKKNKYVYAAIGDPMPKIAGIAKLDVSVAEADRRECIVACRLFGEGCFGGEPFFVAKDPNNSAADEDDGYVVSYVHNEKTGESRFLVMDAKSPNLDIVTAVKLPRRVPYGFHGLFVRETDLRKL

SEQ ID NO: 3 - protein, 601 aa, Nicotiana tabacum
MDAFSSTFLSTLSQHPKSLLSPNYSPNTSSSPILKVSSVRIEERPQTTTTTTRTKPQEKPTPSPYTPPKDTPKRQLPTKSITTKKPVEPSFPSVIFNAFDDFVNTFIDPPLKPCVDPKYILSNNFAPVDELPPTECEVVVGSLPPCLDGAYIRNGPNPQYLPRGPYHLFDGDGMLHSIKISQSKATLCSRYVKTYKYTIEREAGSPVFPNVFSGFNGLTASAARGAITAARAIAGQFNPTNGIGLANTSLALFGGKLFALGESDLPYAVKLAPDGDIITLGRYDFDGKLFMSMTAHPKIDPDTNEAFAFRYGPMPPFLTYFRIEPNGTKTPDVPIFSMTRPSFLHDFAITNKFAIFSDIQIGMNPLEFITGGSPVSSDSGKIPRLGVIPRYAKNESEMKWFDVPGINIVHAINAWDEDDGDTIVMVAPNILSVEHTLERMDMIHASVEKVKIDLKSGMVSRQPLSTRNLDFGVINPAYVGKKNKYVYAAIGDPMPKIAGIAKLDVSVAEADRRDCIVACRLFGEGCFGGEPYFVANNSAADEDDGYVVSFVHNEKTGESRFLVMDAKSPNLDIVAAVKLPRRVPYGFHGLFVRETDLRKLM

SEQ ID NO: 4 - DNA, 1803 bp, Nicotiana tabacum
atggatgccttctcttccactttcctttctacattatcacaacaccctaaatctcttctttctcctaattattctcccaacacatcatcttctccttctcttaaagtctcctccgttagaattgaagaaaggccacaaaccactactagaacaaaaccacaagaaaagccaaccccatcaccctatactgctccaaaagacactcccaaaagacaattacctacaaaatcaataaccccccaaaaaacagtagagccaccatttccatcggttatcttcaatgcatttgacgatttcgtgaacactttcattgatcctcctttgaaaccttctgtcgatccaaagtatattctttctaacaacttcgctccggtggaggagcttcctcctactgaatgcgaggtagtggtaggctcccttccgccttgccttgacggtgcgtacatccgaaatggccccaatcctcagtatcttccacgtggaccttaccatctttttgatggagatggaatgcttcattccattaaaatttctcaaggcaaagctacactctgcagccgatacgtcaaaacttacaaatacacaattgaacgtgaagctggttctccggttttgccaaatgtattctccggtttcaacggtctcactgcctcggcggcgcgtggtgctatcaccgcggctcgagcgattgcaggacagttcaatcccactaacggcataggcctagcaaacacaagcttggctttattcggaggcaaacttttcgctcttggtgaatctgatttaccgtatgcagtaaaattagccccagatggtgatattattaccctcggccgttacgatttcgacggaaaacttttcatgagcatgacggcacatcccaaaattgacccagatactaacgaggcttttgctttccgttacggtccaatgcctccgtttttaacttactttagaatcgaaccaagtggtacaaaaaccccagacgtgccaatattttctatgacacgtccgtcatttctgcatgactttgcaattacaaagaaatatgcgatattctcggatatacaaataggaatgaacccacttgagttcatcgccggtggttcaccggtgagttccgactcagggaaaattccccgtcttggcgtgattccacgttacgccaaggacgagtcagaaatgaagtggttcgatgtgcccgggtttaatatcgtacatgcaattaatgcgtgggatgaagatgacggggatactatagtgatggtggcgccgaatatattgtcggtggagcatacgctggagagaatggatatgatacatgcgtctgttgagaaagtgaagatagatttgaagagtgggatggtgagcagacatccagtttcgacaaggaatcttgattttggagtcatcaatcctgcttatgttgggaagaagaacaagtatgtatatgcagcgattggagacccaatgccaaagatagcaggcatagcaaaattggacgtatcagtagcagaagctgaccggcgcgattgcatagtggggtgccgattatttggcgaaggctgctttggcggcgagccatattttgtggcaaagaatcctaacaactcggtagcggatgaggacgatggctacgttgtgtcgtatgtgcacaatgagaagacaggagagtcaaggttcttggtcatggatgcaaagtcccctaatcttgacattgtggctgctgtcaaattgcctcgtcgagtgccttacggtttccacgggcttttcgtcagggaaattgatcttagcaaactgtag

SEQ ID NO: 5 - DNA, 1803 bp, Nicotiana tabacum
atggatgccttctcttccactttcctttctacattatcactacaccctaaatctcttctttctcctaattattctcccaacacatcatcttctcttgctcttaaggtctcctccgttagaattgaagaaaggccacaaaccactactagaacaaaaccacaagaaaagccaaccccatcaccctacactcctccaaaagacactcccaaaagacaattacctacaaaatcaacaaccacaaaaaaaacagtaaagccatcatttccatcagttatcttcaatgcatttgacgatttcgtgaacactttcattgatcctcctttgaaaccttccgtcgatccaaagtatattctctctaacaactttgctccggtggatgagcttccccctactgaatgcgaggtcgtggtaggctcccttccgccttgccttgacggcgcgtacatccgaaatggccccaatcctcagtatcttccacgtggaccttaccatctttttgatggagatggaatgcttcattgcattaaaatttctcaaggcaaagctacactctgcagccgatacgtcaaaacttacaaatacataattgaacgtgaagctggttctccggttatcccaaatgtattctctggtttcaacggtctcactgcctcggcggcgcgtggtgctatcaccgcagctcgagcgattgcaggacagttcaatcccactaacggcataggcctagcaaacacaagcttagctttattcggaggcaaacttttcgctcttggtgaatctgatttaccatatgcagtaaaattagccccagatggtgatattattaccctcggccgttacgatttcgacggaaagcttttcatgagcatgacggcacatcccaaaattgacccagacactaacgaagcttttgctttccgttacggtccaatgcctccttttctaacttactttagaatcgaaccaaatggtacaaaaaccccagacgtgccaatattttctatgacacgtccgtcatttctgcatgactttgcaattactaagaaatatgcgatattctcggacatacaaataggaatgaacccacttgagttcatcaccggtggttcaccggtgagttccgactctgggaaagttccccgtcttggcgtgattccacgttacgccaaggacgagtcggaaatgaggtggttcgacgtgcccgggtttaatatcgtacatgcaattaatgcgtgggatgaagatgacggggatactatagtgatggtggcgccgaatatattgtcggtggagcatacgctggagagaatggatatgatacatgcttctgttgagaaagtgaagatagatttgaagagtgggatggtgagcagacatccagtgtcgacaaggaatcttgattttggagtcatcaatccggcttatgttgggaagaagaacaagtacgtatatgcagcgattggagaccctatgccaaagatagcaggcatagcaaaattggacgtatcagtagcagaagctgatcggcgcgaatgcatagtggcgtgccgattatttggagaaggctgctttggcggtgagccattttttgtggcaaaggatcccaacaattcggcagcggatgaggacgatggctacgttgtgtcgtatgtgcacaatgagaagacaggagagtcaaggttcttggtcatggatgcaaagtcccctaatcttgacattgtgactgctgtcaaattgcctcgtcgagtgccttacggtttccacggccttttcgtcagggaaactgatcttaggaaactgtag

SEQ ID NO: 6 - DNA, 1806 bp, Nicotiana tabacum
atggatgccttctcttccactttcctttctacattatcacaacaccctaaatctcttctttctcctaattattctcccaacacatcatcttctcctattcttaaggtctcctccgttagaattgaagaaaggccacaaacaactacaaccactactagaaccaaaccacaagaaaagccaaccccatcaccctacactcctccaaaagacactcccaaaagacaattacctacaaaatcaataaccacaaaaaaaccagtagagccatcgtttccatcagttatcttcaatgcatttgacgatttcgtgaacactttcattgatcctcctttgaaaccttgtgtcgatccaaagtatattctctctaacaactttgctccggtggatgagcttccccccactgaatgcgaggtcgtggtaggctcccttcctccttgccttgacggcgcgtacatccgaaatggccccaatcctcagtatcttccacgtggaccttaccatctttttgatggagatggaatgcttcattccattaaaatttctcaaagcaaagctacactctgcagccgatacgtcaaaacttacaaatacacaattgaacgtgaagctggttctccggttttcccaaatgtattctccggtttcaacggtctcactgcctcggcggcgcgtggtgctatcaccgcggctcgagcgattgcgggacagttcaatcccactaacggcatagggctagcaaacacaagcttggctttattcggaggcaaactattcgctcttggtgaatctgatttaccgtatgcagtaaaattagccccagatggtgatattattaccctcggccgttacgatttcgacggaaaacttttcatgagcatgacggcacatcccaaaattgacccagatactaacgaggcttttgctttccgttacggtccaatgcctccttttttaacttactttagaatcgaaccaaatggtacaaaaacaccagacgtgccaatattttctatgacacgtccgtcatttcttcatgactttgcaattacaaataaatttgcgatattctcggacatacaaataggaatgaacccacttgagttcatcaccggtggttcaccggtgagttcagactcggggaaaatccctcgccttggcgtgattccacgttacgccaagaacgaatcggaaatgaagtggtttgatgtgcccgggatcaatattgtacatgcgattaatgcgtgggatgaagatgatggtgatactatagtgatggtagcgcctaatatattgtcggtggagcatacgctggagagaatggatatgatacatgcttctgttgagaaagtgaagatagatttgaagagtgggatggtgagcagacaaccattgtcgacaagaaatcttgattttggagtcatcaatccggcttatgttgggaagaagaacaagtatgtatatgcagcgattggagaccctatgccaaagatagcaggcatagcaaaattggacgtatcagtagcagaagctgatcggcgcgattgcatagtggcgtgccgattatttggagaaggctgctttggcggtgagccatattttgtggcaaacaattcagcagcggatgaggacgatggctacgttgtgtcgtttgtgcacaatgagaagacaggagagtcaaggttcttggtcatggatgcaaagtcccctaatcttgacattgtggctgctgtcaaattgcctcgtcgagtgccttacggtttccacggccttttcgttagggaaactgatcttaggaaactcatgtag

SEQ ID NO: 7 - protein, 600 aa, Nicotiana sylvestris
MDAFSSTFLSTLSQHPKSLLSPNYSPNTSSSPSLKVSSVRIEERPQTTTRTKPQEKPTPSPYTAPKDTPKRQLPTKSITPKKTVEPPFPSVIFNAFDDFVNTFIDPPLKPSVDPKYILSNNFAPVEELPPTECEVVVGSLPPCLDGAYIRNGPNPQYLPRGPYHLFDGDGMLHSIKISQGKATLCSRYVKTYKYTIEREAGSPVLPNVFSGFNGLTASAARGAITAARAIAGQFNPTNGIGLANTSLALFGGKLFALGESDLPYAVKLAPDGDIITLGRYDFDGKLFMSMTAHPKIDPDTNEAFAFRYGPIPPFLTYFRIEPSGTKTPDVPIFSMTRPSFLHDFAITKKYAIFSDIQIGMNPLEFIAGGSPVSSDSGKIPRLGVIPRYAKDESEMKWFDVPGFNIVHAINAWDEDDGDTIVMVAPNILSVEHTLERMDMIHASVEKVKIDLKSGMVSRHPVSTRNLDFGVINPAYVGKKNKYVYAAIGDPMPKIAGIAKLDVSVAEADRRDCIVGCRLFGEGCFGGEPYFVAKNPNNSVADEDDGYVVSYVHNEKTGESRFLVMDAKSPNLDIVAAVKLPRRVPYGFHGLFVREIDLSKL

SEQ ID NO: 8 - DNA, 1803 bp, Nicotiana sylvestris
atggatgccttctcttccactttcctttctacattatcacaacaccctaaatctcttctttctcctaattattctcccaacacatcatcttctccttctcttaaagtctcctccgttagaattgaagaaaggccacaaaccactactagaacaaaaccacaagaaaagccaaccccatcaccctatactgctccaaaagacactcccaaaagacaattacctacaaaatcaataacccccaaaaaaacagtagagccaccatttccatcggttatcttcaatgcatttgacgatttcgtgaacactttcattgatcctcctttgaaaccttctgtcgatccaaagtatattctttctaacaacttcgctccggtggaggagcttcctcctactgaatgcgaggtagtggtaggctcccttccgccttgccttgacggtgcgtacatccgaaatggccccaatcctcagtatcttccacgtggaccttaccatctttttgatggagatggaatgcttcattccattaaaatttctcaaggcaaagctacactctgcagccgatacgtcaaaacttacaaatacacaattgaacgtgaagctggttctccggttttgccaaatgtattctccggtttcaacggtctcactgcctcggcggcgcgtggtgctatcaccgcggctcgagcgattgcaggacagttcaatcccactaacggcataggcctagcaaacacaagcttggctttattcggaggcaaacttttcgctcttggtgaatctgatttaccgtatgcagtaaaattagccccagatggtgatattattaccctcggccgttacgatttcgacggaaaacttttcatgagcatgacggcacatcccaaaattgacccagatactaacgaggcttttgctttccgttacggtccaatacctccgtttttaacttactttagaatcgaaccaagtggtacaaaaaccccagacgtgccaatattttctatgacacgtccgtcatttctgcatgactttgcaattacaaagaaatatgcgatattctcggatatacaaataggaatgaacccacttgagttcatcgccggtggttcaccggtgagttccgactcagggaaaattccccgtcttggcgtgattccacgttacgccaaggacgagtcagaaatgaagtggttcgatgtgcccgggtttaatatcgtacatgcaattaatgcgtgggatgaagatgacggggatactatagtgatggtggcgccgaatatattgtcggtggagcatacgctggagagaatggatatgatacatgcgtctgttgagaaagtgaagatagatttgaagagtgggatggtgagcagacatccagtttcgacaaggaatcttgattttggagtcatcaatcctgcttatgttgggaagaagaacaagtatgtatatgcagcgattggagacccaatgccaaagatagcaggcatagcaaaattggacgtatcagtagcagaagctgaccggcgcgattgcatagtggggtgccgattatttggcgaaggctgctttggcggcgagccatattttgtggcaaagaatcctaacaactcggtagcggatgaggacgatggctacgttgtgtcgtatgtgcacaatgagaagacaggagagtcaaggttcttggtcatggatgcaaagtcccctaatcttgacattgtggctgctgtcaaattgcctcgtcgagtgccttacggtttccacgggcttttcgtcagggaaattgatcttagcaaactgtag

SEQ ID NO: 9 - DNA, 24 bp, Artificial sequence
  Synthetic primer
caccgcgtacatccgaaatggccc

SEQ ID NO: 10 - DNA, 20 bp, Artificial Sequence
  Synthetic primer
agtttgcctccgaataaagc

SEQ ID NO: 11 - DNA, 323 bp, Artificial sequence
  Synthetic: RNAi trigger sequence derived from Nicotiana tabacum
gcgtacatccgaaatggccccaatcctcagtatcttccacgtggaccttaccatctttttgatggagatggaatgcttcattccattaaaatttctcaaagcaaagctacactctgcagccgatacgtcaaaacttacaaatacacaattgaacgtgaagctggttctccggttttcccaaatgtattctccggtttcaacggtctcactgcctcggcggcgcgtggtgctatcaccgcggctcgagcgattgcgggacagttcaatcccactaacggcatagggctagcaaacacaagcttggctttattcggaggcaaact

SEQ ID NO: 12 - DNA, 21 bp, Artificial Sequence
  Synthetic primer
tcatcttctccttctcttaaa

SEQ ID NO: 13 - DNA, 19 bp, Artificial Sequence
  Synthetic primer
cggagaatacatttggcaa

SEQ ID NO: 14 - DNA, 21 bp, Artificial Sequence
  Synthetic primer
tcatcttctcttgctcttaag

SEQ ID NO: 15 - DNA, 19 bp, Artificial Sequence
  Synthetic primer
cagagaatacatttgggat

SEQ ID NO: 16 - DNA, 26 bp, Artificial Sequence
  Synthetic primer
cctttctacattatcacaacacccta

SEQ ID NO: 17 - DNA, 20 bp, Artificial Sequence
  Synthetic primer
tcaccatctggggctaattt

SEQ ID NO: 18 - DNA, 4940 bp, Nicotiana tabacum
agatgaacatggaagattgtatctcttgtgtatctttcgtatatcccttgtatatcaaatacatatatcttgtgtatctcatgtatatccacgtaaaccttaatgtgagatacgtgtttcatttatatgtcaggaaaaaaattttaaactcgatttcaactacaaattttgattataaattagtccaagtaacttccaatcttcctcgaattatgcatattgactcatctatatattttcaatgaatttcaaccatacccattatatatatatattttcttcgtgcttcgtcaacatttcctttatgtcttacatttaatattgcagatacagtaacaacatcatacacagtatattctcacaagtaaagtctggggcatttaatattgcagatcatgcttaaaatataaaaggaggtttttgcgcgtgattacggagggaaagaatccttatatatctggaaatttcaatttctatatacacttagctaaaggtgtattattaatggttaaaggttggcaaggttttgacttattttagatatttccacatgatcactctcaattaaaaactgcctcaagccccttcttcataaaattaaaaggactttttggacaatttggaaaaaagatatttagatgttccgtatttgttgggttttagaatttataagctttaagcgatgtgaatatgtattaatcgacaggtgactatttatcaaaactaagtgtcataattaaacgccttatttcgtccggtgaatagaaacttaggtgttgtgtagatgaggagtctcttttcattgccccacgtcaggaaaatgtggtgttccctaaatgaatagtccctttcgtttgccttactagttactactcactcttatcccacatactgtataaactggccatgggacctcagttcatgcaagaacttattatattcctttactctttagtatcacatcttgtttcttcttttcttcaagacaagaagaaacataatggatgccttctcttccactttcctttctacattatcacaacaccctaaatctcttctttctcctaattattctcccaacacatcatcttctccttctcttaaagtctcctccgttagaattgaagaaaggccacaaaccactactagaacaaaaccacaagaaaagccaaccccatcaccctatactgctccaaaagacactcccaaaagacaattacctacaaaatcaataaccccccaaaaaacagtagagccaccatttccatcggttatcttcaatgcatttgacgatttcgtgaacactttcattgatcctcctttgaaaccttctgtcgatccaaagtatattctttctaacaacttcgctccggtggaggagcttcctcctactgaatgcgaggtagtggtaggctcccttccgccttgccttgacggtgcgtacatccgaaatggccccaatcctcagtatcttccacgtggaccttaccatctttttgatggagatggaatgcttcattccattaaaatttctcaaggcaaagctacactctgcagccgatacgtcaaaacttacaaatacacaattgaacgtgaagctggttctccggttttgccaaatgtattctccggtttcaacggtctcactgcctcggcggcgcgtggtgctatcaccgcggctcgagcgattgcaggacagttcaatcccactaacggcataggcctagcaaacacaagcttggctttattcggaggcaaacttttcgctcttggtgaatctgatttaccgtatgcagtaaaattagccccagatggtgatattattaccctcggccgttacgatttcgacggaaaacttttcatgagcatgacggcacatcccaaaattgacccagatactaacgaggcttttgctttccgttacggtccaatgcctccgtttttaacttactttagaatcgaaccaagtggtacaaaaaccccagacgtgccaatattttctatgacacgtccgtcatttctgcatgactttgcaattacaaagaaatatgcgatattctcggatatacaaataggaatgaacccacttgagttcatcgccggtggttcaccggtgagttccgactcagggaaaattccccgtcttggcgtgattccacgttacgccaaggacgagtcagaaatgaagtggttcgatgtgcccgggtttaatatcgtacatgcaattaatgcgtgggatgaagatgacggggatactatagtgatggtggcgccgaatatattgtcggtggagcatacgctggagagaatggatatgatacatgcgtctgttgagaaagtgaagatagatttgaagagtgggatggtgagcagacatccagtttcgacaaggaatcttgattttggagtcatcaatcctgcttatgttgggaagaagaacaagtacgtataaatcttatcagcaacttataaattaattagatcataaataaattggcataattaatagagtaatgacagtgaaaagaacttttacacagttatgtcacctgaaaacatatttatatacaactattcataattagtcggtagtggcatagcaataatttttattaagaaaggtcaaaatacaaaggaactccgataaaaaagcctagggtattagtatatatatacaaatttatctagctacacgctataaattggacaaaccacttgacactatcagaaatttattggttgggctccatctatagtctagtatatatggccatgtaggtcctactgatcacatgattcatcagatctcacaaaccaaatcatctataattagctattcctcacaggcaaaggcatcttttccccactaaaaatgtactatgttcttctaaatataccaaatatgttaagttcccatcttccaagtaaattatccatgaaaaagtttacaaaatatttgagcaaagaccaaaaatatcatattagtttgtgtactttgtaagccatgcttataatctttcttatttcagtttaaatatctaagcgacaagaatagttataagttcactttgagaaactatatttcttatgaggaaagaacagtttagttgtttggtgaggatccattggcgtgcaagtatcctatgctccaatatgacaatcaaccccaaaaagtaacaaaaggaggagagaagaaaaatctgagattctccaccagttcactgccccacccctttatggatgaaatatgcacatatatataaaatgagtttaagttatatacgtcattaatgtaacggatttttctatcaaataattaaactcatactccgaaccacatataattaggtaacaagcacagaggttgcaccttcagctatagatatggcgggcgaaaaaacaaaagatagacataaatgcaccctagggtgtgacttaattaattgttaataaagttagtaaaactcacaaaagaccaaaatccaaactccagtggagataaaagaaaataaaaggtgatttctcatcatgtatttaagtagtataattaatgtgatttcaatttttactactccaacaggtatgtatatgcagcgattggagacccaatgccaaagatagcaggcatagcaaaattggacgtatcagtagcagaagctgaccggcgcgattgcatagtggggtgccgattatttggcgaaggctgctttggcggcgagccatattttgtggcaaagaatcctaacaactcggtagcggatgaggacgatggctacgttgtgtcgtatgtgcacaatgagaagacaggagagtcaaggttcttggtcatggatgcaaagtcccctaatcttgacattgtggctgctgtcaaattgcctcgtcgagtgccttacggtttccacgggcttttcgtcagggaaattgatcttagcaaactgtagatatatacggatattttatttaaaagtggcaatataagcagtgacggagataccctttacagagagtgtgtgggtgtcatctaactagctgcttcataaaacatcttccttgtgtatatatctatatttaaattattttatatgtatatatagataatagctagttatcataatataatttaaatattgatttgagacaagaaataaaatctcaaaaccaacatattctttcctctccgtgctagttaattatggctatgttcatacttgtctcctaatgatctcccctccggatcccccacaacaacccaattataaaaagacaatatccagacttccagtaagctgaagatgatttctaccaaactgaacatgtggcagaatgattttcttgaatttccgtgtggaatataaaattactgatttgaatggttaatatatatcactacttcaacttaccacctatcgtaataataggcgattttacgacttataattcatttaagtaaatgattattttttttaatttccggctaatttctgggagttgggacagaagtttcggatgaggaatattcacattgtcaaatgtcgtgtaaatttaaagctgtaagctttgttttgttttttaaagagcccatattagcatataccaatacctgtgtctttaagacaacttattggacttggacatgaacatcactactagagtcatagtcttaactattaattaattgtgatcgatacccccagatctaattcaaaaaatctaaaaataaaaagaaaattcagaaaatcttgccaagtggtacatcgaatcaataatagaaatctgttgaattaaatgtggggcgtggcaaggcataagcgttaagacgcaggcaaaaatcccatgttttttttaaaaaaatattttataacttaatacttaacttctttataatttattaagtttaagtttattaagaaattaaactagtcgttaccaattttaaataa

SEQ ID NO: 19 - DNA, 5599 bp, Nicotiana tabacum
  misc_feature (4815)..(4841): n is a, c, g, or t
  misc_feature (5496)..(5599): n is a, c, g, or t
ctcaactccaagattagaagaattacttaccccgaacaagccaaatccaatgccgagaaagctaaacaatgctccacaaatccctctatgtgcgtatcaacttccaaacggcccgaatctagtcaaaataatttgattcagcccacaaaaattataggaattaattccatatcaaaatactaatattttttaaaaatctaaaattgcgccccaaatatcacccgtggggcccacgtctcgaaatccggtaaaaattacaaaaatctgaacccccattcaaccacgagtccaaccataccaaaattactcaaatccgaccacaactcgactttcaaatcctcaatttaaactaagagggttttcaaacttttccaacttaattcaccaattaaatgataaaaacaaccattgattcgggtaatttaaccaatattgagttaagaacacttaccccgttgtttcctctgaaaatcgcccaaaaatcgcctcaatccgagctccaaatcgttaaaaatggaacttaaactttctgaacttaagctttttgtccaggcctctcttcttcgtgaacgcgataggtccctcgcgttcgcgaatcacaactcgactgcccacaaatttaactcttcgcgaacgcaaagctttgcaaatcttactcttcgcgaacgcgaccatggcttcacgaacgcgaagctttactagctcagaccttcgcgaacgcgaacgccacctcgcgaacgcgtagaacaagaacctggggtccccaatcgcctcactcctcttcgcgaacgcgatacctctcacgcgttcgcgatgcgcacacagaccataccttcgcgttacacccgggtgttacaccctttcctttgccttactactcactcttatcccacatacggtataaattggccatgggacctcagttcatgcaagcacttattttattcctttactctttagtatcaaatcttgcttcttcttttcttcaagaagagacataatggatgccttctcttccactttcctttctacattatcactacaccctaaatctcttctttctcctaattattctcccaacacatcatcttctcttgctcttaaggtctcctccgttagaattgaagaaaggccacaaaccactactagaacaaaaccacaagaaaagccaaccccatcaccctacactcctccaaaagacactcccaaaagacaattacctacaaaatcaacaaccacaaaaaaaacagtaaagccatcatttccatcagttatcttcaatgcatttgacgatttcgtgaacactttcattgatcctcctttgaaaccttccgtcgatccaaagtatattctctctaacaactttgctccggtggatgagcttccccctactgaatgcgaggtcgtggtaggctcccttccgccttgccttgacggcgcgtacatccgaaatggccccaatcctcagtatcttccacgtggaccttaccatctttttgatggagatggaatgcttcattgcattaaaatttctcaaggcaaagctacactctgcagccgatacgtcaaaacttacaaatacataattgaacgtgaagctggttctccggttatcccaaatgtattctctggtttcaacggtctcactgcctcggcggcgcgtggtgctatcaccgcagctcgagcgattgcaggacagttcaatcccactaacggcataggcctagcaaacacaagcttagctttattcggaggcaaacttttcgctcttggtgaatctgatttaccatatgcagtaaaattagccccagatggtgatattattaccctcggccgttacgatttcgacggaaagcttttcatgagcatgacggcacatcccaaaattgacccagacactaacgaagcttttgctttccgttacggtccaatgcctccttttctaacttactttagaatcgaaccaaatggtacaaaaaccccagacgtgccaatattttctatgacacgtccgtcatttctgcatgactttgcaattactaagaaatatgcgatattctcggacatacaaataggaatgaacccacttgagttcatcaccggtggttcaccggtgagttccgactctgggaaagttccccgtcttggcgtgattccacgttacgccaaggacgagtcggaaatgaggtggttcgacgtgcccgggtttaatatcgtacatgcaattaatgcgtgggatgaagatgacggggatactatagtgatggtggcgccgaatatattgtcggtggagcatacgctggagagaatggatatgatacatgcttctgttgagaaagtgaagatagatttgaagagtgggatggtgagcagacatccagtgtcgacaaggaatcttgattttggagtcatcaatccggcttatgttgggaagaagaacaagtacgtataaatctcatcagcaacttaattaattagatcataagtaaattggcataattagtagagtttaaatgatagtaaaaaagaacttttacacaattatgttacctaaaaagataattacagccaactcttcataattaatggaccagcaacttaaaaaataaggctgttaattaacttgctatgaattttaaaagataatataaacagttagtgtatacagttaacatcaattaaatgtacttgttactccctccgttctggtttatataaacttatttcctttttggtccattccaaaaagaatgatccatttctaaatttggaaacaatttagcttaaacttacaattctacccttaatgacaagtatttaacttgtttaagaccacaaattccaaaaatctttattttttcttaaacttcatgcccattcaaacatgttcacataaattggaacagagggagagggagtactagattggacttaaacgtctttaaagagaattggaaatatggaaatagtattacaaattataataaatcatcatagaaatcaagcatgttcatggatgtgcttatttgcaacattaaatttttcgatgttatatgaaactgagacatgaaatatctcaccttaacgcgttaatcactaagtcaaggattcattgacagtttagttaggtaattgttgacatgaaaatttaaaacttataatggattagaatatgagatggaatacaatgtttttgtagcattgaaattttaatacaattgagaaaataatcgaaaatcggaagtacttatcgtgttaatggggtcacaagtgtaaaaatattcaaagtaaataaaatatttggtttaaatataaaggagataaatagcaggctggctaaaaggtacagtaaaaaattaacatgagcttaattaagtaaaatccaataaacaaaaatgtcattttagggttgacatagatattttgtttatgtgatatagctcagtagtttcataattaggacaaaccacttgacactatcagaaatttattggttgggctccatctacagactatagtctagcatggccatttaggtcctactgatcacttgattcagcagatatcacaaaccaaactattctaataagcaattccccacaggcaaaggcagcttttccccactcttaaaatatacttttgtctacatgttcttctaaacataccaaatatgttaagttcccatcttccaagtaaattatccatgaaaaagtttacaaaatattttagtaaggaccaaaaatatcatttcagtttgtgtactttgtaagccatgccttataatctttcttatttcagtttaaatatctaagtgacaagaatagttataagttcactttgaaactgaaacacaacatcctttgagaaactgtattccttacgaggaaagaacagtgtagttgtttggtgagggtccattggcgtacaagtagcctatgctgcaatatgacaatcaaccccaaaaagtaacaaaaggaggagagaagaaaaatctaagattctccaccagttcagaaataatactagatacggtggggaaaaaactagagagagatagctatgcacccaagtgtgtgacttaattaattgttaaaaaagttagtaaaactcacaaaacaccaacatccaaactccagtggagataaaagaaaatataaggtgatttctcatcatgtatttaaatagtacgtataatttaggtagaaaattaatgtgatttcattttcactactccaacaggtacgtatatgcagcgattggagaccctatgccaaagatagcaggcatagcaaaattggacgtatcagtagcagaagctgatcggcgcgaatgcatagtggcgtgccgattatttggagaaggctgctttggcggtgagccattttttgtggcaaaggatcccaacaattcggcagcggatgaggacgatggctacgttgtgtcgtatgtgcacaatgagaagacaggagagtcaaggttcttggtcatggatgcaaagtcccctaatcttgacattgtgactgctgtcaaattgcctcgtcgagtgccttacggtttccacggccttttcgtcagggaaactgatcttaggaaactgtagatatatacggatattttgttttaaaagtggcaatataggcagtgacggagatatataccttttagagagggtatgggtgtcatctaaaacttcttccttgtatatatatgtatatttaaattattttatatgtatatatagataatagctagttatgataatattattttaatattgaattgacacaacaaataaatatcaaaaccaaccgattnnnnnnnnnnnnnnnnnnnnnnnnnnncccccccccccccacacacacacacaccacacacatccaattaaaagaagacattatccagacttccagtaagctgaagctgatttctaccaaactgaacattgattttcttgaattttcctgtggaatataaaattactgatttgaattttcgtgtggaatatagaattgccaagtggtacatcgaatcaataatagaaatctattgaattaattgtggggcgtggcaaggcgtaagcgttaaggcgcagggtgcccttgatttttaattttttataacttaataaaataattatataaataaagttcgtaattagctacttagaggcctagttcaaatagaattcttcctaaaaggtggttgtgtagattaattgctcttctttagctgtttttcaaaagacttgtatttatatgtgaaatatgatatttctactaaataaactaaaagacttttagccttgaattttttgtaaattatcttacttagttacttcatagtttggggttatattaaataattacaagtcttttatatctattaaaatatttcgttgcaagtctttcttttaatattttataatttcttacttagcttctttaaaatttattaagtttaagtttattaagaaactagtcttatcaattttaaatnnnnnnnnnnnnnnnnnnnnnnnnnnnnnnnnnnnnnnnnnnnnnnnnnnnnnnnnnnnnnnnnnnnnnnnnnnnnnnnnnnnnnnnnnnnnnnnnnnnnnnnn

SEQ ID NO: 20 - DNA, 5448 bp, Nicotiana tabacum
gttaaatattcataaaagtttccaaggaacaaatcaaaaagaatccaaaaatatttttttgcactgtatttgagtaatttttgcgtagttcctacacttttctgcattatttctgcattcttggtgcacaatttctgcataattcctacgtttttctgctatgttttatattatttctgcattttttctgtactctttttgcatatagtttctgcagttttttgcacaatttctgcatagtttttgcatttttctgcattgattctgcactcttttgcatagtttctatatttgttttgtatatttctacactattttagcttcagtttatgtacttcttttgcaacagtgcagcaacaatataattttcttgcatcttggatgatatgaagtaatgtctttgagtatttgaatttagtataataagaaaatattgttggatggagttttctgttaagaaaaatattgtttgtataagtcatgaaatatctaaggttaaaataggaaatagaatttatccaactttaaaccaaacacatgttttggattatatatggtactccctccattccaatttatgtgaacggcacggagtttaagaaaaaataagacttttggaatttgtgattttaaataattcaaaaagggtctagagtatttgtgtggttataaaagcttctcattaagggtagaattgtaagtttaagccagattgtttccaaatttaaaaaaagatcattctttttggaacagacaaaaaagaactctcgcattgcgcagatgaggagtctcttttcattgccccacgttaggaaaatgtggtgttccctaaacgaatagtccccttcctttgccttaatactcactcttaagtcttatcccacatactgtataaattggccatgggacctcagttcatgacttcattcaagcacttattttattcctttactctttagtatcaaatcttgtttcttcttttcttcaagaagaaacataatggatgccttctcttccactttcctttctacattatcacaacaccctaaatctcttctttctcctaattattctcccaacacatcatcttctcctattcttaaggtctcctccgttagaattgaagaaaggccacaaacaactacaaccactactagaaccaaaccacaagaaaagccaaccccatcaccctacactcctccaaaagacactcccaaaagacaattacctacaaaatcaataaccacaaaaaaaccagtagagccatcgtttccatcagttatcttcaatgcatttgacgatttcgtgaacactttcattgatcctcctttgaaaccttgtgtcgatccaaagtatattctctctaacaactttgctccggtggatgagcttccccccactgaatgcgaggtcgtggtaggctcccttcctccttgccttgacggcgcgtacatccgaaatggccccaatcctcagtatcttccacgtggaccttaccatctttttgatggagatggaatgcttcattccattaaaatttctcaaagcaaagctacactctgcagccgatacgtcaaaacttacaaatacacaattgaacgtgaagctggttctccggttttcccaaatgtattctccggtttcaacggtctcactgcctcggcggcgcgtggtgctatcaccgcggctcgagcgattgcgggacagttcaatcccactaacggcatagggctagcaaacacaagcttggctttattcggaggcaaactattcgctcttggtgaatctgatttaccgtatgcagtaaaattagccccagatggtgatattattaccctcggccgttacgatttcgacggaaaacttttcatgagcatgacggcacatcccaaaattgacccagatactaacgaggcttttgctttccgttacggtccaatgcctccttttttaacttactttagaatcgaaccaaatggtacaaaaacaccagacgtgccaatattttctatgacacgtccgtcatttcttcatgactttgcaattacaaataaatttgcgatattctcggacatacaaataggaatgaacccacttgagttcatcaccggtggttcaccggtgagttcagactcggggaaaatccctcgccttggcgtgattccacgttacgccaagaacgaatcggaaatgaagtggtttgatgtgcccgggatcaatattgtacatgcgattaatgcgtgggatgaagatgatggtgatactatagtgatggtagcgcctaatatattgtcggtggagcatacgctggagagaatggatatgatacatgcttctgttgagaaagtgaagatagatttgaagagtgggatggtgagcagacaaccattgtcgacaagaaatcttgattttggagtcatcaatccggcttatgttgggaagaagaacaagtacgtataaatctcatcaccaacttaattaattagatcataagtaaattggcataattagtagagtttaaatgacagtaaaaaggaacttttacacaattatgttcataattaatggataattacagacaagtcatcataattaatggatcagcaaggcagttaacttgctatgaacattaaaagattgtaattagcaacatcaattaaatttaactgttactagattggaagtaaacgtctttaaagagaattggaaatatggatatagtcttacagattataataaatcatcatagaaatcaagcctgttcatggatgtgcttatttgcaaaattaaattttttcgatgttatgtgaaactgagacatgaaatatttcaccttaacgcgttaattaataagtcaaggattcattgacaataaatcaaggattcaaaaacagctgatttgaataaaaatgagttaactaggctaaaaggtaaaaactaaacaagagcctaattaagttaaatccaataaacaaaaatgtcattttaggagtgacagagatagtttgtttataagatactcttccgttcgggacggagattaaaaaaaagaagaaacttttgaatcgtgtggtcttaaagtttaagggtaaaagttttgtaggttcatgatatttatgtggttatagaagctactcattaaagataaaataggtaaaataaaaattttaaaattaattattttcaaagttagaaatatgtgttttattttgaacaaactaaaaactagtttcataaacccacaaatcacttgacactatcagaaatttattggttgggctccatctatagtccagcatggccatgtaggtcctactgaccacatgattcagcagatctcacaaaccaaaccatctatagttagcaattcctcacaggcaaaggcagcttttccccactaaaaatgtacgtttgtctacatgttcttctaaacataccaaatatgttaagttcccatcttccaagtaaattatccatgaataagtatacaaaatatttgagtaaagaccaaaatatcatttcaattgtaagccatgcttataatctttcttatttcagtttaaatatctaagtgacaagaatagttataagttcactttgaaattgaaatacaacatcctttgagcaactgtattaattccttatgaggaaagaacagtttagttgtttggtgaggatccattggcgtccaagtaccctatgctgcaatatgacaatcaacctcaaaaagtaacaaaaggaggagagatgaaaaatccaaggttttcacccgttcaccgcccccaacccttaatttatggatgaaatatgcacatgtatataaaatgagtttatgttatatatatcattagtgtacgtaaaggatttttctatcaaataaactcatactccgtataaattaggtaacaagcagaaaggttgcacctaaattaattgttaataaagttagtaaaattctcaaaagaccaaaatccaaactccagcggagataaaagaattaaaatataagatgatttcttatcatgtatttaatatatataatttaggtagaaaattaattaatgtgatttcataatttttactactccaacaggtatgtatatgcagcgattggagaccctatgccaaagatagcaggcatagcaaaattggacgtatcagtagcagaagctgatcggcgcgattgcatagtggcgtgccgattatttggagaaggctgctttggcggtgagccatattttgtggcaaacaattcagcagcggatgaggacgatggctacgttgtgtcgtttgtgcacaatgagaagacaggagagtcaaggttcttggtcatggatgcaaagtcccctaatcttgacattgtggctgctgtcaaattgcctcgtcgagtgccttacggtttccacggccttttcgttagggaaactgatcttaggaaactcatgtagtgtagatatatatatatacccatcgatatataccttttagagagggtgtcggtgtcattcaacgctgcttcataaaacatcttccttgtatatgtacgtatatttaaataattttatatgtatatatagataaataatagctagttatcataatagtgatttgagacaagaaataaaatcgcatattgtttcctctccctgctagttatggttacgttcatacttgtctcctaatcctcccccccaaacacccaattaaaagaagacattatccagacttccagtaagctgaagatgatttcgattttctaccaaactgaacatgtggcagaacattgattttcttgaattttcgggtggaagaaatggttaatatatatcactagttcaacttaacgcctatcgtaatgataaaacttataactcatttaagaaaatattttttttattattttccggctaatttctgggagttgggacaaaagttttcggatgaggaatactcttattgtcaaatgttatgtagtgtaaatttagaagctgtaagctttgttttgatttttaaagactccatattagcatatactaatacctgcgtttttaagacaacatattggacttggacatgagcatcactactagagtcatagtcttaactcttaagtaattgtgatcgatacctaggtatggtaaatgggacggtgcgagtgcgggcggtgcggtgcggtgcggtttttaggttatgcggggcgggggcgggggcgggggcggggcgtgttgaggtaattttttttaaaattggtgcgggcagggcggattgcgggtctatgtggatttacgcgggtttaagcaacttttgtggttggcttattctgcaaattatccaccaaacagaaacctagatataagattaaaaataaggtaaactttctaacaaaatagtaaaagctatttaaaattcttaaccaaatttagtatttcatattatcttagagaatgg

SEQ ID NO: 21 - DNA, 4935 bp, Nicotiana sylvestris
gatgaacatggaagattgtatctcttgtgtatctttcgtatatcccttgtatatcaaatacatatatcttgtgtatctcatgtatatccacgtaaaccttaatgtgagatacgtgtttcatttatatgtcaggaaaaaaattttaaacttgatttcaactacaaattttgattataaattagtccaagtaacttccattcttcctcgaattatgcatattgactcatctatatattttcaatgaatttcaaccatacccattatatatatatattttcttcgtgcttcgtcaacatttcctttatgtcttacatttaatattgcagatacagtaacaacatcatacacagtatattctcacaagtaaagtctggggcatttaatattgcagatcacgcttaaaatataaaaggaggtttttgcgcgtgattacggagggaaagaatccttatatatctggaaatttcaatttctatatacacttagctaaaggtgtattattaatggttaaaggttggcaaggttttgacttattttagatatttccacatgatcactctcaattaaaaactgcctcaagccccttcttcataaaattaaaaggactttttggacaatttggaaaaaagatatttagatgttccgtatttgttgggttttagaatttataagctttaagcgatgtgaatatgtattaatcgacaggtgactatttatcaaaactaagtgtcataattaaacgccttatttcgtccggtgaatagaaacttaggtgttgtgtagatgaggagtctcttttcattgccccacgtcaggaaaatgtggtgttccctaaatgaatagtccctttcgtttgccttactagttactactcactcttatcccacatactgtataaactggccatgggacctcagttcatgcaagaacttattatattcctttactctttagtatcacatcttgtttcttcttttcttcaagacaagaagaaacataatggatgccttctcttccactttcctttctacattatcacaacaccctaaatctcttctttctcctaattattctcccaacacatcatcttctccttctcttaaagtctcctccgttagaattgaagaaaggccacaaaccactactagaacaaaaccacaagaaaagccaaccccatcaccctatactgctccaaaagacactcccaaaagacaattacctacaaaatcaataacccccaaaaaaacagtagagccaccatttccatcggttatcttcaatgcatttgacgatttcgtgaacactttcattgatcctcctttgaaaccttctgtcgatccaaagtatattctttctaacaacttcgctccggtggaggagcttcctcctactgaatgcgaggtagtggtaggctcccttccgccttgccttgacggtgcgtacatccgaaatggccccaatcctcagtatcttccacgtggaccttaccatctttttgatggagatggaatgcttcattccattaaaatttctcaaggcaaagctacactctgcagccgatacgtcaaaacttacaaatacacaattgaacgtgaagctggttctccggttttgccaaatgtattctccggtttcaacggtctcactgcctcggcggcgcgtggtgctatcaccgcggctcgagcgattgcaggacagttcaatcccactaacggcataggcctagcaaacacaagcttggctttattcggaggcaaacttttcgctcttggtgaatctgatttaccgtatgcagtaaaattagccccagatggtgatattattaccctcggccgttacgatttcgacggaaaacttttcatgagcatgacggcacatcccaaaattgacccagatactaacgaggcttttgctttccgttacggtccaatacctccgtttttaacttactttagaatcgaaccaagtggtacaaaaaccccagacgtgccaatattttctatgacacgtccgtcatttctgcatgactttgcaattacaaagaaatatgcgatattctcggatatacaaataggaatgaacccacttgagttcatcgccggtggttcaccggtgagttccgactcagggaaaattccccgtcttggcgtgattccacgttacgccaaggacgagtcagaaatgaagtggttcgatgtgcccgggtttaatatcgtacatgcaattaatgcgtgggatgaagatgacggggatactatagtgatggtggcgccgaatatattgtcggtggagcatacgctggagagaatggatatgatacatgcgtctgttgagaaagtgaagatagatttgaagagtgggatggtgagcagacatccagtttcgacaaggaatcttgattttggagtcatcaatcctgcttatgttgggaagaagaacaagtacgtataaatcttatcagcaacttataaattaattagatcataaataaattggcataattaatagagtaatgacagtgaaaagaacttttacacagttatgtcacctgaaaacatatttatatacaactattcataattagtcggtagtggcatagcaataatttttattaagaaaggtcaaaatacaaaggaaataaaaaagcctagggtattagtatatatatacaaatttatctagctacacgctataaattggacaaaccacttgacactatcagaaatttattggttgggctccatctatagtctagtatatatggccatgtaggtcctactgatcacatgattcatcagatctcacaaaccaaatcatctataattagctattcctcacaggcaaaggcatcttttccccactaaaaatgtactatgttcttctaaatataccaaatatgttaagttcccatcttccaagtaaattatccatgaaaaagtttacaaaatatttgagtaaagaccaaaaatatcatattagtttgtgtactttgtacgccatgcttataatctttcttatttcagtttaaatatctaagcgacaagaatagttataagttcactttgagaaactatatttcttatgaggaaagaacagtttagttgtttggtgaggatccattggcgtgcaagtatcctatgctccaatatgacaatcaaccccaaaaagtaacaaaaggaggagagaagaaaaatctgagattctccaccagttcactgccccacccctttatggatgaaatatgcacatatatataaaatgagtttaagttatatacgtcattaatgtaacggatttttctatcaaataattaaactcatactccgaaccacatataattaggtaacaagcacagaggttgcaccttcagctatagatatggcggccgaaaaaacaaaagatagacataaatgcaccctagggtgtgacttaattaattgttaataaagttagtaaaactcacaaaagaccaaaatccaaactccagtggagataaaagaaaataaaaggtgatttctcatcatgtatttaagtagtataattaatgtgatttcaatttttactactccaacaggtatgtatatgcagcgattggagacccaatgccaaagatagcaggcatagcaaaattggacgtatcagtagcagaagctgaccggcgcgattgcatagtggggtgccgattatttggcgaaggctgctttggcggcgagccatattttgtggcaaagaatcctaacaactcggtagcggatgaggacgatggctacgttgtgtcgtatgtgcacaatgagaagacaggagagtcaaggttcttggtcatggatgcaaagtcccctaatcttgacattgtggctgctgtcaaattgcctcgtcgagtgccttacggtttccacgggcttttcgtcagggaaattgatcttagcaaactgtagatatatacggatattttatttaaaagtggcaatataagcagtgacggagataccctttacagagagtgtgtgggtgtcatctaactagctgcttcataaaacatcttccttgtgtatatatctatatttaaattattttatatgtatatatagataatagctagttatcataatataatttaaatattgatttgagacaagaaataaaatctcaaaaccaacatattctttcctctccgtgctagttaattatggctatgttcatacttgtctcctaatgatctcccctccggatcccccacaacaacccaattataaaaagacaatatccagacttccagtaagctgaagatgatttctaccaaactgaacatgtggcagaatgattttcttgaattttcgtgtggaatataaaattactgatttgaatggttaatatatatcactacttcaacttaccacctatcgtaataataggcgattttacgacttataattcatttaagtaaatgattattttttttaatttccggctaatttctgggagttgggacagaagtttcggatgaggaatattcacattgtcaaatgtcgtgtaaatttaaagctgtaagctttgttttgttttttaaagagcccatattagcatataccaatacctgtgtctttaagacaacttattggacttggacatgaacatcactactagagtcatagtcttaactattaattaattgtgatcgatacccccagatctaattcaaaaaatctaaaaataaaaagaaaattcagaaaatcttgccaagtggtacatcgaatcaataatagaaatctgttgaattaaatgtggggcgtggcaaggcataagcgttaagacgcaggcaaaaatcccatgttttttttaaaaaaatattttataacttaatacttaacttctttataatttattaagtttaagtttattaagaaattaaactagtcgttaccaattttaaataat

SEQ ID NO: 22 - DNA, 18 bp, artificial sequence
  Synthetic primer
caaactccagcggagata

SEQ ID NO: 23 - DNA, 18 bp, artificial sequence
  Synthetic primer
ggcacgccactatgcaat